European Patent Specification EP 3 735 464 B1, published March 15, 2023. Title: Regeneration of genetically modified plants. Applicant: KWS SAAT SE BASF SE. The sequence listing filed with the application follows.

SEQUENCE LISTING (210 sequences)

SEQ ID NO: 1 - DNA, 1194 bp, Artificial Sequence
  cDNA of AtGRF5
atgatgagtctaagtggaagtagcgggagaacaataggaaggcctccatttacaccaacacaatgggaagaactggaacatcaagccctaatctacaagtacatggtctctggtgttcctgtcccacctgagctcatcttctccattagaagaagcttggacacttccttggtctctagactccttcctcaccaatcccttggatgggggtgttaccagatgggatttgggagaaaaccagatccagagccaggaagatgcagaagaacagatggtaagaaatggagatgctcaagagaagcttacccagattcgaagtactgtgaaaaacacatgcacagaggaagaaaccgtgccagaaaatctcttgatcagaatcagacaacaacaactcctttaacatcaccatctctctcattcaccaacaacaacaacccaagtcccaccttgtcttcttcttcttcctctaattcctcttctactacttattctgcttcttcttcttcaatggatgcctacagtaacagtaataggtttgggcttggtggaagtagtagtaacactagaggttatttcaacagccattctcttgattatccttatccttctacttcacccaaacaacaacaacaaactcttcatcatgcttccgctttgtcacttcatcaaaatactaattctacttctcagttcaatgtcttagcctctgctactgaccacaaagacttcaggtactttcaagggattggggagagagttggaggagttggggagagaacgttctttccagaagcatctagaagctttcaagattctccataccatcatcaccaacaaccgttagcaacagtgatgaatgatccgtaccaccactgtagtactgatcataataagattgatcatcatcacacatactcatcctcatcatcatctcaacatcttcatcatgatcatgatcatagacagcaacagtgttttgttttgggcgccgacatgttcaacaaacctacaagaagtgtccttgcaaactcatcaagacaagatcaaaatcaagaagaagatgagaaagattcatcagagtcgtccaagaagtctctacatcacttctttggtgaggactgggcacagaacaagaacagttcagattcttggcttgacctttcttcccactcaagactcgacactggtagctaa

SEQ ID NO: 2 - protein, 397 aa, Arabidopsis thaliana
MMSLSGSSGRTIGRPPFTPTQWEELEHQALIYKYMVSGVPVPPELIFSIRRSLDTSLVSRLLPHQSLGWGCYQMGFGRKPDPEPGRCRRTDGKKWRCSREAYPDSKYCEKHMHRGRNRARKSLDQNQTTTTPLTSPSLSFTNNNNPSPTLSSSSSSNSSSTTYSASSSSMDAYSNSNRFGLGGSSSNTRGYFNSHSLDYPYPSTSPKQQQQTLHHASALSLHQNTNSTSQFNVLASATDHKDFRYFQGIGERVGGVGERTFFPEASRSFQDSPYHHHQQPLATVMNDPYHHCSTDHNKIDHHHTYSSSSSSQHLHHDHDHRQQQCFVLGADMFNKPTRSVLANSSRQDQNQEEDEKDSSESSKKSLHHFFGEDWAQNKNSSDSWLDLSSHSRLDTGS

SEQ ID NO: 3 - DNA, 1143 bp, Artificial Sequence
  cDNA of BvGRF5
atgagcactgctacagcaacagtaggaggtggtggtggtggaggaagaagtaaattcccatttacagcaacacaatggcaagaacttgaacatcaagctctaatttataagtatatggctgctggtgttcctattcctcctgatcttcttttcaccatcaaacgtagtcttgactcttctctctcctccaagctctttccttaccaaccttctcctttgggatggaacccatatcaaatggggtatggaaaaaagatagacccagaaccaggaaggtgcagaagaacagatgggaaaaaatggaggtgttcaaaagaagcatacccagattcaaagtactgtgagaggcacatgcatagaggcaaaaaccgttcaagaaagcctgtggaatcacctttgactacaacttcaactactgtttctaataacaacaataataataataataataataattctgctgcaaattcatcactgacagtagcagctgctgctgctgcagcatctttgaccaatcaatcactgcttaataagaatccttcttctgtttcaacttctctcttttctcttccttcctctgattcctcttgtaattctcacctcctttatccccattcttcttacaatcacaaggactatagggaaaggtattatcaaggattaaaagaggaggtgggagagcatgcatttttcacagagagctcaggatcaagtatgagaggtttttcaggttcatccatggatgaaagttggcaaattggtggtggaagtaacatagatcatcatcaacaacaacaacaacaatcaaaacaaagtggtgggtaccctaattacttgcagcagcttcaaagtaatagtacaactagtaataatggtacatcagcaaagcaggagaagcaatgctacatttggggaagagattttaactgtgatttatcaatgaaggttgaagaagaaagagaaaactttcatgaaaaaaccacccaccatttctttgatgaatggcctattaaaagtggtggaagaggaggaagagattcttcatggcatgattcttcttcaactactcaactttccatatccattccttcttctacttctcatcatcatgactttttcctcacaaattctagggactcctaa

SEQ ID NO: 4 - protein, 380 aa, Beta vulgaris
MSTATATVGGGGGGGRSKFPFTATQWQELEHQALIYKYMAAGVPIPPDLLFTIKRSLDSSLSSKLFPYQPSPLGWNPYQMGYGKKIDPEPGRCRRTDGKKWRCSKEAYPDSKYCERHMHRGKNRSRKPVESPLTTTSTTVSNNNNNNNNNNNSAANSSLTVAAAAAAASLTNQSLLNKNPSSVSTSLFSLPSSDSSCNSHLLYPHSSYNHKDYRERYYQGLKEEVGEHAFFTESSGSSMRGFSGSSMDESWQIGGGSNIDHHQQQQQQSKQSGGYPNYLQQLQSNSTTSNNGTSAKQEKQCYIWGRDFNCDLSMKVEEERENFHEKTTHHFFDEWPIKSGGRGGRDSSWHDSSSTTQLSISIPSSTSHHHDFFLTNSRDS

SEQ ID NO: 5 - DNA, 1197 bp, Artificial Sequence
  cDNA of ZmGRF5
atgatgatgatgagcagcggccgggcgggcggcggggccaccgcggggcggtacccgttcacggcgtcgcagtggcaggagctggagcaccaggcgctcatctacaagtgcctggcgtccggcaagcccatcccttcctacctcatgccgccgctccgccgcatcctcgactccgccctcgccacgtcgccgtccctcgcctacccgccgcaaccctcactgggctggggctgcttcgggatgggcttcacccggaaggccgacgaggacccggagcccgggcggtgccggcgcacggacggcaagaagtggcgctgctccaaggaggcgtacccggactccaagtactgcgagaagcacatgcaccggggcaagaaccgttcaagaaagcctgtggaaatgtccttggccacgccggccccggcgccggcccccgccgccgccacaaccgccaccgccacctcatccccggcgccgtcctaccaccgcccggcccacgacgccacgccgtctccgtaccacgcgctgtatggaggcggcggcggcggcggcggtagcccttactcggcgtcggcacgcccaggagcaaccggaggcggcggcgcgtaccaccacgcgcagcatgtgagccccttccacctccacctcgagaccacccacccgcacccgccgccgccctacaactactccgccgaccagagggactacgcgtacgggcacgcggccgccaaggaggtcggcgagcacgccttcttctcggacggcgcgggcgagcgggtcgaccggcaggccgcggcggggcagtggcagttcaggcagctcggggtggagacgaagccgggccccacgccgctgttccccgtcgccgggtacgggcacggcgcggcgtcgccgtacggcgtggagatgggcaaggacgacgacgagcaggaggagaggcgccgccagcactgcttcgttcttggagccgacctgcggctggagcggccgtcgtcgggccatggccatggccatgaccatgacgacgccgccgccgcgcagaagccgctccggcccttcttcgacgagtggccgcaccagaagggggacaaggccgggtcgtggatggggctcgacggcgagacgcagctctccatgtccatccccatggccgccaccgacctccccgtcacctcccgcttccgtaacgacgagtga

SEQ ID NO: 6 - protein, 398 aa, Zea mays
MMMMSSGRAGGGATAGRYPFTASQWQELEHQALIYKCLASGKPIPSYLMPPLRRILDSALATSPSLAYPPQPSLGWGCFGMGFTRKADEDPEPGRCRRTDGKKWRCSKEAYPDSKYCEKHMHRGKNRSRKPVEMSLATPAPAPAPAAATTATATSSPAPSYHRPAHDATPSPYHALYGGGGGGGGSPYSASARPGATGGGGAYHHAQHVSPFHLHLETTHPHPPPPYNYSADQRDYAYGHAAAKEVGEHAFFSDGAGERVDRQAAAGQWQFRQLGVETKPGPTPLFPVAGYGHGAASPYGVEMGKDDDEQEERRRQHCFVLGADLRLERPSSGHGHGHDHDDAAAAQKPLRPFFDEWPHQKGDKAGSWMGLDGETQLSMSIPMAATDLPVTSRFRNDE

SEQ ID NO: 7 - DNA, 1245 bp, Artificial Sequence
  cDNA of TaGRF5
atgatgatgatgggtggtcgcgcgggggccggcggcgtcggggcaggcggggggcggtgcccgttcacggcgacgcagtggcaggagcttgagcaccaggcactcatctacaagtacatggcctccggcgtgcccatcccctccgacctcctcctcccgctccgccgcagcttcctcctcgactccgccctcgccacctccccctccctcgccttccctccccaggccgcacttggctggggttgctttggcatggggttcggccggaaggcggaggacccggagccggggcggtgccggcggacggacggcaagaagtggcgctgctccaaggaggcgtacccggactccaagtactgcgagaagcacatgcaccgcggcaagaaccgttcaagaaagcctgtggaaatgtccttggccacgcccccgccgccgccttcctcctcggcctcctcctcctcctccaacgtccactccgccgtcaacgtcgccaccaccacctcctcccccgcgccgtcctaccaccgccacgccgccgcgactcacgacacgacgccctaccacgcgctctacggcggcccctactcctccgccggccgccagcagcacgctagcgcctaccaccacgccgcgcaggtcagcccgttccacctgcacctcgacaccacccacccgcacccgccgccgtcctactactccagcatggaccacagcaaggacagctacgcctacgggcacagcgtcaaggaggtgcacggcggcggcgagcacgccttcttctcctccgacgtcaccaccgacagggaccatcaccaccaccaccatcagcaccaacaccacgctagcgccggcggcaacggccagtggcagttcaagcagctcggcggcatggagccgaagcagcataacccaacgtcgctcttccccggctgcggcggctacggcaacaacgcggcctacgccatcgacctgtccagcaaagaagaggacgaggagaaggagaggcggcagcagcagcagcactgcttcctgctgggcgccgacctgaggctcgacaagccgtcgtcggggcacggcgactccgccgaccagaagcctctccggcccttcttcgacgagtggccgcacgagaagaccgggagcaaggggtcgtggatggggctcgagggggagacgcagctctccatctccatcgccaacgaactccccatcaccaccacctcccgctaccaccatggtgaatga

SEQ ID NO: 8 - protein, 414 aa, Triticum aestivum
MMMMGGRAGAGGVGAGGGRCPFTATQWQELEHQALIYKYMASGVPIPSDLLLPLRRSFLLDSALATSPSLAFPPQAALGWGCFGMGFGRKAEDPEPGRCRRTDGKKWRCSKEAYPDSKYCEKHMHRGKNRSRKPVEMSLATPPPPPSSSASSSSSNVHSAVNVATTTSSPAPSYHRHAAATHDTTPYHALYGGPYSSAGRQQHASAYHHAAQVSPFHLHLDTTHPHPPPSYYSSMDHSKDSYAYGHSVKEVHGGGEHAFFSSDVTTDRDHHHHHHQHQHHASAGGNGQWQFKQLGGMEPKQHNPTSLFPGCGGYGNNAAYAIDLSSKEEDEEKERRQQQQHCFLLGADLRLDKPSSGHGDSADQKPLRPFFDEWPHEKTGSKGSWMGLEGETQLSISIANELPITTTSRYHHGE

SEQ ID NO: 9 - DNA, 1170 bp, Artificial Sequence
  cDNA of BnGRF5
atgatgagtctaagtggaaatggtgggagaacaatagagaggcctccatttacaccaacacaatggcaagaactggagaatcaagccctaatttacaagtacatggtctcaggagttcctgtcccacctgagctcatcttctccattagaagaagcttggactcttccttggtctctagactcctccctcaccaatccattgggtggggatgctatcagatggggtttggtagaaaaccagatccagaaccaggaaggtgcagaagaacagatggtaagaaatggagatgctcaagagaagcatacccagattcaaagtactgtgaaaaacacatgcacagaggaaggaaccgtgccagaaaatctattgatcagaatcagacaactgctcctttaacatcaccatctctctctttccccaacaacaacaacccaagccctaccttgtcttcttcctcctctacttattcagctgcttcttcatctccttccattgatgcttacagtaatatcaataggcttggtgttggtagtagtaacagtagaggttacttcaacaaccattcccttgactatccttatcctttgtcctcacctaaacagcaacaacaacagactcttcatcatgcttctgctttgtctcttcaccaaaacacatctactgattctcagttcaatgccttagcttctgcaactgaccataaagacttcagatactttcaagggattggggagagagctggagttggagctggggagaggactttttttccagaagcttctagaagctttcaagattctccataccatcaccaacgaccgttagcaacagtaatgaatgacccgtaccactctggtactgatcataaggttgatcatcatcatcacacatactcatccgtatcatcatcatctcagcatgatcaagatcatcatcgacaacaacagcagcaatgttttgttatgggcgctgacatgttcaacaaacccacaagaactgtcttcgcaaacacatcgaggcaagatcatcaagaagaggaggagaaagattcatcagaaacaaagaagtctctacatcatttctttggtgaggactgggcgcagaacaaaaacaattcagattcttggcttgacctttcttcccattcaagactcgacactggtagttga

SEQ ID NO: 10 - protein, 389 aa, Brassica napus
MMSLSGNGGRTIERPPFTPTQWQELENQALIYKYMVSGVPVPPELIFSIRRSLDSSLVSRLLPHQSIGWGCYQMGFGRKPDPEPGRCRRTDGKKWRCSREAYPDSKYCEKHMHRGRNRARKSIDQNQTTAPLTSPSLSFPNNNNPSPTLSSSSSTYSAASSSPSIDAYSNINRLGVGSSNSRGYFNNHSLDYPYPLSSPKQQQQQTLHHASALSLHQNTSTDSQFNALASATDHKDFRYFQGIGERAGVGAGERTFFPEASRSFQDSPYHHQRPLATVMNDPYHSGTDHKVDHHHHTYSSVSSSSQHDQDHHRQQQQQCFVMGADMFNKPTRTVFANTSRQDHQEEEEKDSSETKKSLHHFFGEDWAQNKNNSDSWLDLSSHSRLDTGS

SEQ ID NO: 11 - DNA, 1173 bp, Artificial Sequence
  cDNA of BrGRF5
atgatgagtctaagtggaaatggtgggagaacaatagagaggcctccatttacaccaacacaatggcaagaactggagaatcaagccctaatttacaagtacatggtctcaggagttcctgtcccacctgagctcatcttctccattagaagaagcttggactcttccttggtctctagactcctccctcaccaatccattgggtggggatgctatcagatggggtttggtagaaaaccagatccagaaccaggaaggtgcagaagaacagatggtaagaaatggagatgctcaagagaagcacatccagattctaagtactgtgaaaaacacatgcacagaggaaggaaccgtgccagaaaatctattgatcagaatcagacaactgctcctttaacatcaccatctctctctttccccaacaacaacaacccaagccctaccttgtcttcttcctcctctacttattcagcttcttcttcatctccttccattgatgcttacagtaatatcaataggcttggtgttggtaatagtaacagtagaggttacttcaacaaccattcccttgactatccttatcctttgtcctcacctaaacagcaacaacaacaacagactcttcatcatgcttctgctttgtctcttcaccaaaacgcatctactgcttctcagttcaatgccttagcttctgcaactgaccataaagacttcagatactttcaagggattggggagagagttggagttggagctggggagaggactttttttccagaagcttctagaagctttcaagattctccataccatcaccaacaaccgttagctacagtaatgaatgacccgttccactctggtactgatcataaggttgatcatcagcatcacacatactcatccgtatcatcatcatctcagcatgatcaagatcatcatcgacaacaacagcagcaatgttttgttatgggcgctgacatgttcaacaaacccacaagaactgtcttcgcaaactcatctagacaagatcatcaagaagaggaggagaaagattcatcagaaacaaagaagtctctacatcatttctttggtgaggactgggcacagaacaaaaacagttcagattcttggcttgacctttcttcccattcaagactggacactggtagttga

SEQ ID NO: 12 - protein, 390 aa, Brassica rapa
MMSLSGNGGRTIERPPFTPTQWQELENQALIYKYMVSGVPVPPELIFSIRRSLDSSLVSRLLPHQSIGWGCYQMGFGRKPDPEPGRCRRTDGKKWRCSREAHPDSKYCEKHMHRGRNRARKSIDQNQTTAPLTSPSLSFPNNNNPSPTLSSSSSTYSASSSSPSIDAYSNINRLGVGNSNSRGYFNNHSLDYPYPLSSPKQQQQQQTLHHASALSLHQNASTASQFNALASATDHKDFRYFQGIGERVGVGAGERTFFPEASRSFQDSPYHHQQPLATVMNDPFHSGTDHKVDHQHHTYSSVSSSSQHDQDHHRQQQQQCFVMGADMFNKPTRTVFANSSRQDHQEEEEKDSSETKKSLHHFFGEDWAQNKNSSDSWLDLSSHSRLDTGS

SEQ ID NO: 13 - DNA, 1173 bp, Artificial Sequence
  cDNA of BoGRF5
atgatgagtctaagtggaaatggtgggagaacaatagagaggcctccatttacaccaacacaatggcaagaactggagaatcaagccctaatttacaagtacatggtctcaggagttcctgtcccacctgagctcatcttctccattagaagaagcttggactcttccttggtctctagactcctccctcaccaatccattgggtggggatgctatcagatggggtttggtagaaaaccagatccagaaccaggaaggtgcagaagaacagatggtaagaaatggagatgctcaagagaagcataccctgattcaaagtactgtgaaaaacacatgcacagaggaaggaaccgtgccagaaaatctattgatcagaatcagacaactgctcctctaacttcaccatctctctctttccccaacaacaacaacccaagccctaccttgtcctcttcctcctctacttattcagcttcttcttcatctccttccattgatgcttacagtaatatcaataggcttggtgttggtagtagtaacagtagaggttacttcaacaaccattcccttgagtatccttatcctttgtcctcacctaaacagcaacaacaacaacagactcttcatcatgcttctgctttgtctcttcaccaaaacacatctactgcttctcagttcaatgccttagcttctgcaaccgaccataaagacttcagatattttcaagggattggggagagagttggagttggagctggggagagaactttttttccagaagcttctagaagctttcaagattctccataccatcaccaacaaccgttagcaacagtaatgagtgacccgtaccactctggtactgatcataaggttgatcatcatcctcacacatactcatccgtatcatcatcatctcagcatgatcaagatcatcatcgacaacaacagcagcaatgttttgttatgggcgctgacatgttcaacaaacccacaagaactggcttcgcaaacacatcgaggcaagatcatcaagaagaggaggagaaagattcatcagaaacaaagaagtctctacatcatttctttggtgaggactgggcgcagaacaaaaacaattcagattcttggcttgacctttcttcccattcaagactcgacactggtagttga

SEQ ID NO: 14 - protein, 390 aa, Brassica oleracea
MMSLSGNGGRTIERPPFTPTQWQELENQALIYKYMVSGVPVPPELIFSIRRSLDSSLVSRLLPHQSIGWGCYQMGFGRKPDPEPGRCRRTDGKKWRCSREAYPDSKYCEKHMHRGRNRARKSIDQNQTTAPLTSPSLSFPNNNNPSPTLSSSSSTYSASSSSPSIDAYSNINRLGVGSSNSRGYFNNHSLEYPYPLSSPKQQQQQQTLHHASALSLHQNTSTASQFNALASATDHKDFRYFQGIGERVGVGAGERTFFPEASRSFQDSPYHHQQPLATVMSDPYHSGTDHKVDHHPHTYSSVSSSSQHDQDHHRQQQQQCFVMGADMFNKPTRTGFANTSRQDHQEEEEKDSSETKKSLHHFFGEDWAQNKNNSDSWLDLSSHSRLDTGS

SEQ ID NO: 15 - DNA, 1197 bp, Artificial Sequence
  cDNA of RsGRF5
atgatgagtctaagtggaaatggtgggagaacaatagagaggcctccatttacaccaacacaatggcaagaactggagagtcaagccctaatttacaagtacatggtctcaggggttcctgtcccacctgagctcatcttctccattagaagaagcttggactcttccttggtctctagactcctccctcaccaatctcttggctggggatgctatcagatgggatttggtagaaaaccagatccggaaccaggaaggtgcagaagaacagatggtaagaaatggagatgctcaagagaagcatacccagattcaaagtactgtgaaaaacacatgcacagaggaaggaaccgtgccaggaaatctattgatcagaatcagacaactgctcctttgacatcaccatctctctctttccccaacaacccaagccctaccttgtcttcttcttcttctgcctctacttattctgctgcatcttcatctccttctattgatgctttcagtaatatcaataggcctggtgttggtagtagcatcagcagaggttacttcaacaaccattcccttgactatccttatcctttgtcctcacctaaacaacaacagcaacaacagactcttcatcatgcttctgctttgtcacttcaccaaaacacatctactgcttctcagttcaatgtcttagcctcttcaactgaccataaagacttcagatactttcaagggattggggagagagttggagttggagttggggagagaacattttttccagaagcttctagaagctttcaagattctccataccatcaccaacaaccgttggcaacagtaatgaatgacccgtaccactgtagtactgatcacaaggttgatcatcatcacacatactcatccgcatcatcatcgtctcaacatcaacatgatcaagatcatgagcatagacaacaacagcagcaatgtttcgttatgggtgctgacatgttcaacaaacccacacgaactgtcttcgcaaacacatcgagacaagatcaagaagaggaggagaaagattcatctgaaaccaagaagtctctacatcatttctttggtgaggactgggcgcagaacaagaacagttcagattcttggcttgatctttcttcccactcaagactcgaccctggtagtaacctacattctgatctatgctaa

SEQ ID NO: 16 - protein, 398 aa, Raphanus sativus
MMSLSGNGGRTIERPPFTPTQWQELESQALIYKYMVSGVPVPPELIFSIRRSLDSSLVSRLLPHQSLGWGCYQMGFGRKPDPEPGRCRRTDGKKWRCSREAYPDSKYCEKHMHRGRNRARKSIDQNQTTAPLTSPSLSFPNNPSPTLSSSSSASTYSAASSSPSIDAFSNINRPGVGSSISRGYFNNHSLDYPYPLSSPKQQQQQQTLHHASALSLHQNTSTASQFNVLASSTDHKDFRYFQGIGERVGVGVGERTFFPEASRSFQDSPYHHQQPLATVMNDPYHCSTDHKVDHHHTYSSASSSSQHQHDQDHEHRQQQQQCFVMGADMFNKPTRTVFANTSRQDQEEEEKDSSETKKSLHHFFGEDWAQNKNSSDSWLDLSSHSRLDPGSNLHSDLC

SEQ ID NO: 17 - DNA, 1182 bp, Artificial Sequence
  cDNA of SbGRF5
atgatgatgatgagcggtcgagcgggcggcggcgccaccgcggggcggtacccgttcacggcgtcgcagtggcaggagctggagcaccaggcgctcatctacaagtgcctggcgtctggcaagcccatcccgtcctacctcatgccgccgctccgccgcatcctcgactccgccctcgccacgtcgccgtccctcgccttcccgccgcaaccctcgttggggtggggctgtttcgggatgggcttcagcaggaagcccgacgaggacccggagcccggccggtgccggcggacggacggcaagaagtggcgctgctccaaggaggcgtacccggactccaagtactgcgagaagcacatgcaccggggcaagaaccgttcaagaaagcctgtggaaatgtccttggccacaccggcgccggcctctgcggtgtcctccgccacaagcgccacagccgccgccgccgccgccaccaccaccacctcgtcgccagcaccgtcctaccgcccagcgcccacctcgcacgacgcctcgccgtaccacgcgctgtacggcggcggcagtccgtactcggcgtcggcgcgtcccgccggtggccccggcccgtaccatcatcccgcgcaggtgagccccttccacctccacctcgagaccacccacccgcacccgccgccgtcctactactccgtagaccagcgggactacgcgtacgggcacgccaccaaggaggtcgtcggcgagcacgccttcttctccgatggcgcggccgagcgggaccgccagcatgccgccggccagtggcagttcaagcagctcgggatggacacgaagccgagccccacgtctctgttccccgtcgccgggtacggcaacggcgctggtgcgtcgccgtacggcgttgatctgggagccaaggaagacgacgaggaagaaaggcggcgccagcagcagcagcactgcttcgttcttggtgccgacctgcggctggagcggccgtcgtcgggccatgacgccgccaccgcgcagaagccgctccggcccttctttgacgagtggccgcacgagaagggaaacaagggtgggtcatggatggggcttgacggcgagacgcagctctccatgtccatccccatggccgccagcgacctccccgtcacctcccgctaccgtaatgatgagtga

SEQ ID NO: 18 - protein, 393 aa, Sorghum bicolor
MMMMSGRAGGGATAGRYPFTASQWQELEHQALIYKCLASGKPIPSYLMPPLRRILDSALATSPSLAFPPQPSLGWGCFGMGFSRKPDEDPEPGRCRRTDGKKWRCSKEAYPDSKYCEKHMHRGKNRSRKPVEMSLATPAPASAVSSATSATAAAAAATTTTSSPAPSYRPAPTSHDASPYHALYGGGSPYSASARPAGGPGPYHHPAQVSPFHLHLETTHPHPPPSYYSVDQRDYAYGHATKEVVGEHAFFSDGAAERDRQHAAGQWQFKQLGMDTKPSPTSLFPVAGYGNGAGASPYGVDLGAKEDDEEERRRQQQQHCFVLGADLRLERPSSGHDAATAQKPLRPFFDEWPHEKGNKGGSWMGLDGETQLSMSIPMAASDLPVTSRYRNDE

SEQ ID NO: 19 - DNA, 1002 bp, Artificial Sequence
  cDNA of HaGRF5
atgatgagtacaacagcaggtgaaggtgtaaggaatcatagtggaaggtatcccttcacagccactcaatggcaagaacttgaacatcaagcacttgtttacaaatacatgatctctggtatgcctatcccccctgatctgcttttcaccatcaaaacaagtctagattcttctacaaagctcctccttcaccaccagccacctcatccctcctcaattggatggaactgcttccagatgggatttgggagaaaaatagatccagaaccaggaagatgcagaagaacagatggtaagaaatggaggtgttcaaaagaagcctatcctgattcaaaatactgtgaaaggcacatgcacagaggcagaaaccgttcaagaaagcctgtggaagtcaacatgtcgtcaacaccaacacccaaaacaccaccaaccgccattccaatgatcccatcttccatctgtaccaaatccccaaattacccttctcccaattcacatccactctcttcttcttcttctgactattaccataataataacaccacccaccttccatcttattctagaccttcttctaatgttttcacacaagaccacttcttgttggattctagcccatacatgagaaaggggtatgggatgaaagaggtgatagatgagcactcatttttctcagaatcttctggaaccatcaagactgattcttggcaattggaaccactggctatgaacaattcatcctcaaagcaaacaactttttctgattatcatcaaaacagatactcatatcaacaacagcaagatccaggctattatgatcaacaactggctttgaaaattgacagaaatgatgaaccccagaaagtaatgcaccatttctttgatgaatggccaccaaatgatgataataacaaagattcttcttccactactcagctctcaatatccatccccagttctgctcgtgatttcttcctctcacataatgctggtgataaatga

SEQ ID NO: 20 - protein, 333 aa, Helianthus annuus
MMSTTAGEGVRNHSGRYPFTATQWQELEHQALVYKYMISGMPIPPDLLFTIKTSLDSSTKLLLHHQPPHPSSIGWNCFQMGFGRKIDPEPGRCRRTDGKKWRCSKEAYPDSKYCERHMHRGRNRSRKPVEVNMSSTPTPKTPPTAIPMIPSSICTKSPNYPSPNSHPLSSSSSDYYHNNNTTHLPSYSRPSSNVFTQDHFLLDSSPYMRKGYGMKEVIDEHSFFSESSGTIKTDSWQLEPLAMNNSSSKQTTFSDYHQNRYSYQQQQDPGYYDQQLALKIDRNDEPQKVMHHFFDEWPPNDDNNKDSSSTTQLSISIPSSARDFFLSHNAGDK

SEQ ID NO: 21 - DNA, 1053 bp, Artificial Sequence
  cDNA of StGRF5
atggcggcggagaatgggtacagaccgccgttcacggcggtgcagtggcaggaattggagcatcaagcaatgatatataagtatttggtggcgggtattccggtgccggccgaccttgttgtacctatacgacgtagctttgaacccatttcagcgaggttctttcatcatcctagcttgggttattgctcctattatgggaagaagtttgatcctgagccaggaaggtgtagaaggacagatggaaagaagtggaggtgcgccaaagatgcatatcctgactcaaagtattgcgagcggcacatgcatcgaggccgcaaccgttcaagaaagcatgtggaatctcaatcgactgcccagtccttgttgactagtatgtcacataatactactgggagcagcaaaacaagtggaaacttccaacgtagcagtagtggcaatttccaacgtagcagcagtgaaagcttccagaacacgccactatattctgctgctaatactgaaggaccaagttatggaagtgccacaacaaagatgcagatggagcctgccacctatgcagtagatagcaaggggtatttccatggaatgactgctgatgctgatgagcagaatttctctctcgaagcttcggcaggcacgagaagtttagggatgggatctaacacagacagcatgtggtgtctgatgcctcctccacaacttccctcaagccccatggtgaaaccaaaaaatgattcacagttgctagatagctcgcgacatatccgaatgcctaatccattcgagcctatgaatgatacaactatttcgggacaacaccaacattgctttttcagcagtgacataggctctcccgggacagtaaagcaggagcaacgttcaatgcgccctttctttgacgaatggcctacaactaaggaatcatggtccaatcttgatgatgagggatccaacaaaaataatttctccactactcagctgtccatatccattcctatggctccttctgacttctcttcaaggagttcttgttccccaaacgatgcttga

SEQ ID NO: 22 - protein, 350 aa, Solanum tuberosum
MAAENGYRPPFTAVQWQELEHQAMIYKYLVAGIPVPADLVVPIRRSFEPISARFFHHPSLGYCSYYGKKFDPEPGRCRRTDGKKWRCAKDAYPDSKYCERHMHRGRNRSRKHVESQSTAQSLLTSMSHNTTGSSKTSGNFQRSSSGNFQRSSSESFQNTPLYSAANTEGPSYGSATTKMQMEPATYAVDSKGYFHGMTADADEQNFSLEASAGTRSLGMGSNTDSMWCLMPPPQLPSSPMVKPKNDSQLLDSSRHIRMPNPFEPMNDTTISGQHQHCFFSSDIGSPGTVKQEQRSMRPFFDEWPTTKESWSNLDDEGSNKNNFSTTQLSISIPMAPSDFSSRSSCSPNDA

SEQ ID NO: 23 - DNA, 1242 bp, Artificial Sequence
  cDNA of HvGRF5
atgatgatgatgggcggtcgcgcgggggccggcggcgtgggggcaggcggggggcggtgcccgttcacggcgacgcagtggcaggagctggagcaccaggcgctcatctacaagtacatggcctccggcgtgcctatcccctccgacctcctcctcccgctccgccgcagcttcctcctcgactccgccctcgccacctccccctccctcgccttccctccgcaggccacactgggctggggttgcttcgggatggggttcggccggaagccggaggacccggagccggggcggtgccggcggacggacggcaagaagtggcgctgctccagggaggcgtacccagactccaagtactgcgagaagcacatgcaccgcggcaagaaccgttcaagaaagcctgtggaaatgtccttggccacgcccccgccgccgccttcctcctcggcctcctcctcctcctccaacgtccactccgccgtcaccgtcgccaccaccaccacctcccccgcgccgtcctaccaccgccacgccgccacgactcacgacgcggcaccctaccacgcgctctacggcggcccctacgcctccgccggccgccagcagcacgggagcgcctaccaccacgccgcgcaggtcagcccgttccacctgcacctcgacaccacccacccgcacccgccgccgtcctactactccaccatggaccacagcaaggacagctacgcctacgggcacagcgtcaaggaggtgcacggcggcggcgagcacgccttcttctcctccgacgtcaccaccgacagggaccaccagcaccaccaacaccacggcagcgccggcggccacggccagtggcagttcaagcagctcggcggcatggagccgaagcagcacaaccccacgtcgctcttccccgggtgcggcggctacggcaacaacgcagcgtacgccatcgacctgtccggcaaagaagaggccgaggagaaggagaggcggcagcagcagcagcactgcttcctgctgggcgctgacctgaggctcgacaagccgtcgtcggggcacggcgactccgccgaccagaagcctctccggccgttcttcgacgagtggccgcacgagaagaccgggaacaaggggtcatggatggggctcgagggcgagacccagctctccatctccatccccatgaccgccaacgacctccccatcaccaccacctcccgttaccaccacggtgaatga

SEQ ID NO: 24 - protein, 413 aa, Hordeum vulgare
MMMMGGRAGAGGVGAGGGRCPFTATQWQELEHQALIYKYMASGVPIPSDLLLPLRRSFLLDSALATSPSLAFPPQATLGWGCFGMGFGRKPEDPEPGRCRRTDGKKWRCSREAYPDSKYCEKHMHRGKNRSRKPVEMSLATPPPPPSSSASSSSSNVHSAVTVATTTTSPAPSYHRHAATTHDAAPYHALYGGPYASAGRQQHGSAYHHAAQVSPFHLHLDTTHPHPPPSYYSTMDHSKDSYAYGHSVKEVHGGGEHAFFSSDVTTDRDHQHHQHHGSAGGHGQWQFKQLGGMEPKQHNPTSLFPGCGGYGNNAAYAIDLSGKEEAEEKERRQQQQHCFLLGADLRLDKPSSGHGDSADQKPLRPFFDEWPHEKTGNKGSWMGLEGETQLSISIPMTANDLPITTTSRYHHGE

SEQ ID NO: 25 - DNA, 1236 bp, Artificial Sequence
  cDNA of ScGRF5
atgatgatgatgggcggtcgcgcgggggccggcggcgtcggggcaggcgggggccggtgcccgttcacggcgacgcagtggcaggagctggagcaccaggcgctcatctacaagtacatggcctccggcgtgcccatcccctccgacctcctcctcccgctccgccgcagcttcctcctcgactccgccctcgccacctccccctccctcgccttccctccccaggccgcacttggatggggctgcttcgggatggggttcggccggaaggcggaggacccggagccggggcggtgccggcggacggacggcaagaagtggcgctgctccaaggaggcgtacccggactccaagtactgcgagaagcacatgcaccgcggcaagaaccgttcaagaaagcctgtggaaatgtccttggccacgcccccgccgccgccttcctcctcggcctcctcctcctcctccaacgtccactccgccgtcaacgtcgccaccaccacctcctcccccgcgccatcctaccaccgccacgccgccgcgactcacgacacgacgccctaccacgcgctctacggcggcccctacgcctctgccggccgccagcagcacgccagcgcctaccaccacgccgcgcaggtcagcccgttccacctgcacctcgacaccacccacccgcacccgccgccgtcctactactccaccatggaccacagcaaggacagctacgcctacgggcacagcgtcaaggaggtgcacggcggcggcgagcacgccttcttcgcctccgacgtcgccaccgacagggaccaccaccaccaccaccaacaccacgccggcgccggcggcaacggccaatggcagttcaagcagctcggcggcatggagcccaagcagcataaccccacgtcgctcttccccggctgcggcggctacggcaacaacgcggcgtacgccatcgacctgtccagcaaagaagaggacgaggagaaggagaggcggcagcagcagcagcactgcttcctgctgggcgccgacctgaggctcgacaagccgtcgtcggggcacggcgactccgccgaccagaagcccctccggccgttcttcgacgagtggccgcacgagaaggccgggagcaaggggtcgtggatggggctcgagggggagacgcagctctccatctccatcgccaacgaactccccatcaccaccacctcccgctaccaccatggtgaatga

SEQ ID NO: 26 - protein, 411 aa, Secale cereale
MMMMGGRAGAGGVGAGGGRCPFTATQWQELEHQALIYKYMASGVPIPSDLLLPLRRSFLLDSALATSPSLAFPPQAALGWGCFGMGFGRKAEDPEPGRCRRTDGKKWRCSKEAYPDSKYCEKHMHRGKNRSRKPVEMSLATPPPPPSSSASSSSSNVHSAVNVATTTSSPAPSYHRHAAATHDTTPYHALYGGPYASAGRQQHASAYHHAAQVSPFHLHLDTTHPHPPPSYYSTMDHSKDSYAYGHSVKEVHGGGEHAFFASDVATDRDHHHHHQHHAGAGGNGQWQFKQLGGMEPKQHNPTSLFPGCGGYGNNAAYAIDLSSKEEDEEKERRQQQQHCFLLGADLRLDKPSSGHGDSADQKPLRPFFDEWPHEKAGSKGSWMGLEGETQLSISIANELPITTTSRYHHGE

SEQ ID NO: 27 - DNA, 1083 bp, Artificial Sequence
  cDNA of GmGRF5
atgatgagtgcaagtgcaggtgcaagaaataggtctccgttcacacaaattcagtggcaagagcttgagcaacaagctcttgtttttaagtacatggttacaggaacacctatcccaccagatctcatctactctattaaaagaagtctagacacttcaatttcttcaaggctcttcccacatcatccaattgggtggggatgttttgaaatgggatttggcagaaaagtagacccagagccagggaggtgcagaagaacagatggcaagaaatggagatgttcaaaggaggcatatccagactcaaagtactgtgaaagacacatgcacagaggcagaaaccgttcaagaaagcctgtggaagtttcttcagcaacaagcaccgccacaaacacctcccaaacaatcccatcatcttataccagaaacctttccttgaccaataacagtaaccccaacataacaccaccaccaccaccctcttctttccctttctctcatttgccctcttctatgcctattgatcagtcccaacccttttcccaatcctaccaaaactcttctctcaatcccttcttctactcccaatcaacctcctctagacccccagatgctgattttccaccccaagatgccaccacccaccacctattcatggactctgctggctcttattctcatgatgaaaagaattatagcaggcatgttcatggaataagggaagatgtggatgagagagctttcttcccagaagcatcaggatcagctaggagctatacagactcgtaccaacaactatcaatgagctcctacaagtcctattcaaactccaactttcagaacattaataatgatgccaccaccaacccaagacagcaagagcagcaactacaacaacaacaacactgttttgttttagggacagacttcaaatcaacaaggccaagcaaagagaaagaagctgagacaacaacaggtcagagaccccttcaccgtttctttggggagtggccaccaaagaacacaacaacagattcctggctagatcttgcttccaactccagaatccaaaccgatgaatga

SEQ ID NO: 28 - protein, 360 aa, Glycine max
MMSASAGARNRSPFTQIQWQELEQQALVFKYMVTGTPIPPDLIYSIKRSLDTSISSRLFPHHPIGWGCFEMGFGRKVDPEPGRCRRTDGKKWRCSKEAYPDSKYCERHMHRGRNRSRKPVEVSSATSTATNTSQTIPSSYTRNLSLTNNSNPNITPPPPPSSFPFSHLPSSMPIDQSQPFSQSYQNSSLNPFFYSQSTSSRPPDADFPPQDATTHHLFMDSAGSYSHDEKNYSRHVHGIREDVDERAFFPEASGSARSYTDSYQQLSMSSYKSYSNSNFQNINNDATTNPRQQEQQLQQQQHCFVLGTDFKSTRPSKEKEAETTTGQRPLHRFFGEWPPKNTTTDSWLDLASNSRIQTDE

SEQ ID NO: 29 - DNA, 945 bp, Artificial Sequence
  cDNA of GhGRF5
atgattagtgccagaaataagtaccttttcactccaaatcaatggcaagagcttgaacaccaagctctcatcttcaaatacatggtttcaggagttcctatcccacctcaactcctttattctgtcaaaacaagctttgattcttctttggcttcacacctcttccctcaccaacccacagggtggggctgttttcaggtgggttttggcagaaaaccagacccagagccggggaggtgcaggagaactgatggaaaaaaatggagatgctccaaagaagcttacccagactccaagtactgtgagaggcacatgcatagaggcaggaaccgttcaagaaagcctgtggaagctaattcatcatcatcaacagcaccaccagcaccaccaacaacagcagcagcttccatcctttcaccatctttcccatcaatcaacagtaaccttcccacttcaagttcttctctctctttttctcctatggctactgaaaacttcacccatttcgacccctttctttattctcattcttctacgagacttcatggttcaggcttatcagttccatctcatcatttcctagactctggaactggaattgattaccctcagactgataaactttacaggtatgttcatggaacaagggaaggtgttgatgaaagatctttcttccccgaagcttcagcgagtgtaagagttgtatctgattcttatcagccactgacaatggtccaaagctttggtgacaacaatggttcaaagcaggggcagcaatgcttcgttttaggtactgatatcaagtcagctaagccaatcaagttagaaaaggatgaaggaactcaaaaaccagtccaccaatttttaggggattggacacaagggaacaacaatggttcttggcttgatcttgcatccaattccagggtccaatcagatagttga

SEQ ID NO: 30 - protein, 314 aa, Gossypium hirsutum
MISARNKYLFTPNQWQELEHQALIFKYMVSGVPIPPQLLYSVKTSFDSSLASHLFPHQPTGWGCFQVGFGRKPDPEPGRCRRTDGKKWRCSKEAYPDSKYCERHMHRGRNRSRKPVEANSSSSTAPPAPPTTAAASILSPSFPSINSNLPTSSSSLSFSPMATENFTHFDPFLYSHSSTRLHGSGLSVPSHHFLDSGTGIDYPQTDKLYRYVHGTREGVDERSFFPEASASVRVVSDSYQPLTMVQSFGDNNGSKQGQQCFVLGTDIKSAKPIKLEKDEGTQKPVHQFLGDWTQGNNNGSWLDLASNSRVQSDS

SEQ ID NO: 31 - DNA, 1194 bp, Artificial Sequence
  cDNA of OsGRF5
atgatgatgatgagcggtcgcccgagcggcggcgccggcggaggtcggtacccgttcacggcgtcgcagtggcaggagctggagcaccaggcgctcatctacaagtacatggcgtccgggactcccatcccctccgacctcatcctccccctccgccgcagcttcctcctcgactccgccctcgccacctccccttccctcgccttccctccccaaccttcactggggtggggttgctttggcatggggtttgggcggaaggcggaggacccggagccagggcgatgccggcgtacggacggcaagaagtggcggtgctccaaggaggcgtacccggactccaagtactgcgagaagcacatgcaccgtggcaagaaccgttcaagaaagcctgtggaaatgtccttggccacgccgccgccgccgtcctcctccgccacctccgccgcgtcgaacacctccgccggcgtcgcccccaccaccaccaccacctcctccccggcgccctcctacagccgcccggcgccgcacgacgcggcgccgtaccaggcgctctacggcgggccctacgccgcggccaccgcgcgcacccccgccgccgcggcgtaccacgcgcaggtgagcccgttccacctccagctcgacaccacccacccgcacccgccgccgtcctactactccatggaccacaaggagtacgcgtacgggcacgccaccaaggaggtgcacggcgagcacgccttcttctccgatggcaccgagagggagcaccaccacgccgccgccgggcacggccagtggcagttcaagcagctcggcatggagcccaagcagagcaccacgcctctcttcccgggcgccggctacggccacaccgcggcgtcgccgtacgccattgatctttcaaaagaggacgacgatgagaaagagaggcggcaacagcagcagcagcagcagcagcagcactgcttcctcctgggcgccgacctccgtctggagaagccggcgggccacgaccacgcggcggcggcgcagaaacctctccgccacttcttcgacgagtggccgcatgagaagaacagcaagggctcctggatggggctcgaaggcgagacgcagctgtccatgtccatccccatggccgccaacgacctcccgatcaccaccacctcccgctaccacaatgatgattaa

SEQ ID NO: 32 - protein, 397 aa, Oryza sativa
MMMMSGRPSGGAGGGRYPFTASQWQELEHQALIYKYMASGTPIPSDLILPLRRSFLLDSALATSPSLAFPPQPSLGWGCFGMGFGRKAEDPEPGRCRRTDGKKWRCSKEAYPDSKYCEKHMHRGKNRSRKPVEMSLATPPPPSSSATSAASNTSAGVAPTTTTTSSPAPSYSRPAPHDAAPYQALYGGPYAAATARTPAAAAYHAQVSPFHLQLDTTHPHPPPSYYSMDHKEYAYGHATKEVHGEHAFFSDGTEREHHHAAAGHGQWQFKQLGMEPKQSTTPLFPGAGYGHTAASPYAIDLSKEDDDEKERRQQQQQQQQQHCFLLGADLRLEKPAGHDHAAAAQKPLRHFFDEWPHEKNSKGSWMGLEGETQLSMSIPMAANDLPITTTSRYHNDD

SEQ ID NO: 33 - protein, 530 aa, Arabidopsis thaliana
MDLGVRVSGHETVSSPGQTELGSGFSNKQERSGFDGEDCWRSSKLSRTSTDGFSSSPASAKTLSFHQGIPLLRSTTINDPRKGQEHMLSFSSASGKSDVSPYLQYCRNSGYGLGGMMNTSNMHGNLLTGVKGPFSLTQWAELEQQALIYKYITANVPVPSSLLLSLKKSFFPYGSLPPNSFGWGSFHLGFSGGNMDPEPGRCRRTDGKKWRCSRDAVPDQKYCERHINRGRHRSRKPVEGQNGHNTNAAAAASAAAASTAAAVSKAAAGTSAVAMRGSDNNNSLAAAVGTQHHTNNQSTDSLANRVQNSRGASVFPATMNLQSKETHPKQSNNPFEFGLISSDSLLNPSHKQASYATSSKGFGSYLDFGNQAKHAGNHNNVDSWPEELKSDWTQLSMSIPMAPSSPVQDKLALSPLRLSREFDPAIHMGLGVNTEFLDPGKKTNNWIPISWGNNNSMGGPLGEVLNSTTNSPKFGSSPTGVLQKSTFGSLSNSSSASSTIIGDNNNKNGDGKDPLGPTTLMNTSATAPSL

SEQ ID NO: 34 - protein, 535 aa, Arabidopsis thaliana
MDIGVHVLGSVTSNENESLGLKELIGTKQDRSGFIGEDCLQRSLKLARTTTRAEEEENLSSSVAAAYCKTMSFHQGIPLMRSASPLSSDSRRQEQMLSFSDKPDALDFSKYVGLDNSSNNKNSLSPFLHQIPPPSYFRSSGGYGSGGMMMNMSMQGNFTGVKGPFTLTQWAELEQQALIYKYITANVPVPSSLLISIKKSFYPYGSLPPSSFGWGTFHLGFAGGNMDPEPGRCRRTDGKKWRCSRDAVPDQKYCERHINRGRHRSRKPVEVQSGQNQTAAAASKAVTTPQQPVVAGNTNRSNARASSNRSLAIGSQYINPSTESLPNNRGVSIYPSTVNLQPKESPVIHQKHRNNNNPFEFGHISSDSLLNPNTAKTYGSSFLDFSSNQEKHSGNHNHNSWPEELTSDWTQLSMSIPIASSSPSSTHNNNNAQEKTTLSPLRLSRELDLSIQTDETTIEPTVKKVNTWIPISWGNSLGGPLGEVLNSTTNSPTFGSSPTGVLQKSTFCSLSNNSSVSSPIAENNRHNGDYFHYTT

SEQ ID NO: 35 - protein, 398 aa, Arabidopsis thaliana
MDLQLKQWRSQQQQQHQTESEEQPSAAKIPKHVFDQIHSHTATSTALPLFTPEPTSSKLSSLSPDSSSRFPKMGSFFSWAQWQELELQALIYRYMLAGAAVPQELLLPIKKSLLHLSPSYFLHHPLQHLPHYQPAWYLGRAAMDPEPGRCRRTDGKKWRCSRDVFAGHKYCERHMHRGRNRSRKPVETPTTVNATATSMASSVAAAATTTTATTTSTFAFGGGGGSEEVVGQGGSFFFSGSSNSSSELLHLSQSCSEMKQESNNMNNKRPYESHIGFSNNRSDGGHILRPFFDDWPRSSLQEADNSSSPMSSATCLSISMPGNSSSDVSLKLSTGNEEGARSNNNGRDQQNMSWWSGGGSNHHHHNMGGPLAEALRSSSSSSPTSVLHQLGVSTQAFH

SEQ ID NO: 36 - protein, 380 aa, Arabidopsis thaliana
MDLQLKQWRSQQQNESEEQGSAATKISNFFFDQIQSQTATSAAAAPLPLFVPEPTSSSSFSCFSPDSSNSSSSSRFLKMGNFFSWAQWQELELQALIYRYMLAGASVPQELLLPIKKSLLHQSPMHFLHHPLQHSFPHHQPSWYWGRGAMDPEPGRCKRTDGKKWRCSRDVVAGHKYCDRHIHRGRNRSRKPVETATTTITTTATTTASSFVLGEELGHGPNNNHFFSSGSSQPLHLSHQQSCSSEMKQESNNNKRPYEANSGFSNGRSDDGHILRHFFDDWPRSSDSTSSPMSSSTCHLSISMPGNNTSSDVSLKLSTGNEEEEENMRNNNNEREQMNWWSNGGNHHNNMGGPLAEALRSASSTSSVLHQMGISTQVFH

SEQ ID NO: 37 - protein, 244 aa, Arabidopsis thaliana
MATRIPFTESQWEELENQALVFKYLAANMPVPPHLLFLIKRPFLFSSSSSSSSSSSFFSPTLSPHFGWNVYEMGMGRKIDAEPGRCRRTDGKKWRCSKEAYPDSKYCERHMHRGKNRSSSRKPPPTQFTPNLFLDSSSRRRRSGYMDDFFSIEPSGSIKSCSGSAMEDNDDGSCRGINNEEKQPDRHCFILGTDLRTRERPLMLEEKLKQRDHDNEEEQGSKRFYRFLDEWPSSKSSVSTSLFI

SEQ ID NO: 38 - protein, 365 aa, Arabidopsis thaliana
MDFLKVSDKTTIPYRSDSLFSLNQQQYKESSFGFRDMEIHPHPTPYAGNGLLGCYYYYPFTNAQLKELERQAMIYKYMIASIPVPFDLLVSSPSSASPCNNKNIAGDLEPGRCRRTDGKKWRCAKEVVSNHKYCEKHLHRGRPRSRKHVEPPYSRPNNNGGSVKNRDLKKLPQKLSSSSIKDKTLEPMEVSSSISNYRDSRGSEKFTVLATTEQENKYLNFIDVWSDGVRSSEKQSTTSTPVSSSNGNLSLYSLDLSMGGNNLMGQDEMGLIQMGLGVIGSGSEDHHGYGPYGVTSSLEEMSSWLAPMSTTPGGPLAEILRPSTNLAISGDIESYSLMETPTPSSSPSRVMKKMTSSVSDESSQV

SEQ ID NO: 39 - protein, 493 aa, Arabidopsis thaliana
MRMLLGIPYVDKSVLSNSVLERGKQDKSKLLLVDKCHYELDVEERKEDFVGGFGFGVVENSHKDVMVLPHHHYYPSYSSPSSSSLCYCSAGVSDPMFSVSSNQAYTSSHSGMFTPAGSGSAAVTVADPFFSLSSSGEMRRSMNEDAGAAFSEAQWHELERQRNIYKYMMASVPVPPELLTPFPKNHQSNTNPDVDTYRSGMFSIYADYKNLPLSMWMTVTVAVATGGSLQLGIASSASNNTADLEPWRCKRTDGKKWRCSRNVIPDQKYCERHTHKSRPRSRKHVESSHQSSHHNDIRTAKNDTSQLVRTYPQFYGQPISQIPVLSTLPSASSPYDHHRGLRWFTKEDDAIGTLNPETQEAVQLKVGSSRELKRGFDYDLNFRQKEPIVDQSFGALQGLLSLNQTPQHNQETRQFVVEGKQDEAMGSSLTLSMAGGGMEETEGTNQHQWVSHEGPSWLYSTTPGGPLAEALCLGVSNNPSSSTTTSSCSRSSS

SEQ ID NO: 40 - protein, 431 aa, Arabidopsis thaliana
MKMQSPKMEQEEVEEERMRNKWPWMKAAQLMEFRMQALVYRYIEAGLRVPHHLVVPIWNSLALSSSSNYNYHSSSLLSNKGVTHIDTLETEPTRCRRTDGKKWRCSNTVLLFEKYCERHMHRGRKRSRKLVESSSEVASSSTKYDNTYGLDRYNESQSHLHGTISGSSNAQVVTIASLPSARSCENVIRPSLVISEFTNKSVSHGRKNMEMSYDDFINEKEASMCVGVVPLQGDESKPSVQKFFPEVSDKCLEAAKFSSNRKNDIIARSREWKNMNVNGGLFHGIHFSPDTVLQERGCFRLQGVETDNEPGRCRRTDGKKWRCSKDVLSGQKYCDKHMHRGMKKKHPVDTTNSHENAGFSPLTVETAVRSVVPCKDGDDQKHSVSVMGITLPRVSDEKSTSSCSTDTTITDTALRGEDDDEEYLSLFSPGV

SEQ ID NO: 41 - protein, 38 aa, Artificial Sequence
  variant of the indicator motif
DPEPGRCRRTDGKKWRCSREAYPDSKYCEKHMHRGRNR

SEQ ID NO: 42 - protein, 38 aa, Artificial Sequence
  variant of the indicator motif
DPEPGRCRRTDGKKWRCAREAYPDSKYCEKHMHRGRNR

SEQ ID NO: 43 - protein, 38 aa, Artificial Sequence
  variant of the indicator motif
DPEPGRCRRTDGKKWRCSKEAYPDSKYCEKHMHRGRNR

SEQ ID NO: 44 - protein, 38 aa, Artificial Sequence
  variant of the indicator motif
DPEPGRCRRTDGKKWRCAKEAYPDSKYCEKHMHRGRNR

SEQ ID NO: 45 - protein, 38 aa, Artificial Sequence
  variant of the indicator motif
DPEPGRCRRTDGKKWRCSRDAYPDSKYCEKHMHRGRNR

SEQ ID NO: 46 - protein, 38 aa, Artificial Sequence
  variant of the indicator motif
DPEPGRCRRTDGKKWRCARDAYPDSKYCEKHMHRGRNR

SEQ ID NO: 47 - protein, 38 aa, Artificial Sequence
  variant of the indicator motif
DPEPGRCRRTDGKKWRCSKDAYPDSKYCEKHMHRGRNR

SEQ ID NO: 48 - protein, 38 aa, Artificial Sequence
  variant of the indicator motif
DPEPGRCRRTDGKKWRCAKDAYPDSKYCEKHMHRGRNR

SEQ ID NO: 49 - protein, 38 aa, Artificial Sequence
  variant of the indicator motif
DPEPGRCRRTDGKKWRCSREAHPDSKYCEKHMHRGRNR

SEQ ID NO: 50 - protein, 38 aa, Artificial Sequence
  variant of the indicator motif
DPEPGRCRRTDGKKWRCAREAHPDSKYCEKHMHRGRNR

SEQ ID NO: 51 - protein, 38 aa, Artificial Sequence
  variant of the indicator motif
DPEPGRCRRTDGKKWRCSKEAHPDSKYCEKHMHRGRNR

SEQ ID NO: 52 - protein, 38 aa, Artificial Sequence
  variant of the indicator motif
DPEPGRCRRTDGKKWRCAKEAHPDSKYCEKHMHRGRNR

SEQ ID NO: 53 - protein, 38 aa, Artificial Sequence
  variant of the indicator motif
DPEPGRCRRTDGKKWRCSRDAHPDSKYCEKHMHRGRNR

SEQ ID NO: 54 - protein, 38 aa, Artificial Sequence
  variant of the indicator motif
DPEPGRCRRTDGKKWRCARDAHPDSKYCEKHMHRGRNR

SEQ ID NO: 55 - protein, 38 aa, Artificial Sequence
  variant of the indicator motif
DPEPGRCRRTDGKKWRCSKDAHPDSKYCEKHMHRGRNR

SEQ ID NO: 56 - protein, 38 aa, Artificial Sequence
  variant of the indicator motif
DPEPGRCRRTDGKKWRCAKDAHPDSKYCEKHMHRGRNR

SEQ ID NO: 57 - protein, 38 aa, Artificial Sequence
  variant of the indicator motif
DPEPGRCRRTDGKKWRCSREAYPDSKYCERHMHRGRNR

SEQ ID NO: 58 - protein, 38 aa, Artificial Sequence
  variant of the indicator motif
DPEPGRCRRTDGKKWRCAREAYPDSKYCERHMHRGRNR

SEQ ID NO: 59 - protein, 38 aa, Artificial Sequence
  variant of the indicator motif
DPEPGRCRRTDGKKWRCSKEAYPDSKYCERHMHRGRNR

SEQ ID NO: 60 - protein, 38 aa, Artificial Sequence
  variant of the indicator motif
DPEPGRCRRTDGKKWRCAKEAYPDSKYCERHMHRGRNR

SEQ ID NO: 61 - protein, 38 aa, Artificial Sequence
  variant of the indicator motif
DPEPGRCRRTDGKKWRCSRDAYPDSKYCERHMHRGRNR

SEQ ID NO: 62 - protein, 38 aa, Artificial Sequence
  variant of the indicator motif
DPEPGRCRRTDGKKWRCARDAYPDSKYCERHMHRGRNR

SEQ ID NO: 63 - protein, 38 aa, Artificial Sequence
  variant of the indicator motif
DPEPGRCRRTDGKKWRCSKDAYPDSKYCERHMHRGRNR

SEQ ID NO: 64 - protein, 38 aa, Artificial Sequence
  variant of the indicator motif
DPEPGRCRRTDGKKWRCAKDAYPDSKYCERHMHRGRNR

SEQ ID NO: 65 - protein, 38 aa, Artificial Sequence
  variant of the indicator motif
DPEPGRCRRTDGKKWRCSREAHPDSKYCERHMHRGRNR

SEQ ID NO: 66 - protein, 38 aa, Artificial Sequence
  variant of the indicator motif
DPEPGRCRRTDGKKWRCAREAHPDSKYCERHMHRGRNR

SEQ ID NO: 67 - protein, 38 aa, Artificial Sequence
  variant of the indicator motif
DPEPGRCRRTDGKKWRCSKEAHPDSKYCERHMHRGRNR

SEQ ID NO: 68 - protein, 38 aa, Artificial Sequence
  variant of the indicator motif
DPEPGRCRRTDGKKWRCAKEAHPDSKYCERHMHRGRNR

SEQ ID NO: 69 - protein, 38 aa, Artificial Sequence
  variant of the indicator motif
DPEPGRCRRTDGKKWRCSRDAHPDSKYCERHMHRGRNR

SEQ ID NO: 70 - protein, 38 aa, Artificial Sequence
  variant of the indicator motif
DPEPGRCRRTDGKKWRCARDAHPDSKYCERHMHRGRNR

SEQ ID NO: 71 - protein, 38 aa, Artificial Sequence
  variant of the indicator motif
DPEPGRCRRTDGKKWRCSKDAHPDSKYCERHMHRGRNR

SEQ ID NO: 72 - protein, 38 aa, Artificial Sequence
  variant of the indicator motif
DPEPGRCRRTDGKKWRCAKDAHPDSKYCERHMHRGRNR

SEQ ID NO: 73 - protein, 38 aa, Artificial Sequence
  variant of the indicator motif
DPEPGRCRRTDGKKWRCSREAYPDSKYCEKHMHRGKNR

SEQ ID NO: 74 - protein, 38 aa, Artificial Sequence
  variant of the indicator motif
DPEPGRCRRTDGKKWRCAREAYPDSKYCEKHMHRGKNR

SEQ ID NO: 75 - protein, 38 aa, Artificial Sequence
  variant of the indicator motif
DPEPGRCRRTDGKKWRCSKEAYPDSKYCEKHMHRGKNR

SEQ ID NO: 76 - protein, 38 aa, Artificial Sequence
  variant of the indicator motif
DPEPGRCRRTDGKKWRCAKEAYPDSKYCEKHMHRGKNR

SEQ ID NO: 77 - protein, 38 aa, Artificial Sequence
  variant of the indicator motif
DPEPGRCRRTDGKKWRCSRDAYPDSKYCEKHMHRGKNR

SEQ ID NO: 78 - protein, 38 aa, Artificial Sequence
  variant of the indicator motif
DPEPGRCRRTDGKKWRCARDAYPDSKYCEKHMHRGKNR

SEQ ID NO: 79 - protein, 38 aa, Artificial Sequence
  variant of the indicator motif
DPEPGRCRRTDGKKWRCSKDAYPDSKYCEKHMHRGKNR

SEQ ID NO: 80 - protein, 38 aa, Artificial Sequence
  variant of the indicator motif
DPEPGRCRRTDGKKWRCAKDAYPDSKYCEKHMHRGKNR

SEQ ID NO: 81 - protein, 38 aa, Artificial Sequence
  variant of the indicator motif
DPEPGRCRRTDGKKWRCSREAHPDSKYCEKHMHRGKNR

SEQ ID NO: 82 - protein, 38 aa, Artificial Sequence
  variant of the indicator motif
DPEPGRCRRTDGKKWRCAREAHPDSKYCEKHMHRGKNR

SEQ ID NO: 83 - protein, 38 aa, Artificial Sequence
  variant of the indicator motif
DPEPGRCRRTDGKKWRCSKEAHPDSKYCEKHMHRGKNR

SEQ ID NO: 84 - protein, 38 aa, Artificial Sequence
  variant of the indicator motif
DPEPGRCRRTDGKKWRCAKEAHPDSKYCEKHMHRGKNR

SEQ ID NO: 85 - protein, 38 aa, Artificial Sequence
  variant of the indicator motif
DPEPGRCRRTDGKKWRCSRDAHPDSKYCEKHMHRGKNR

SEQ ID NO: 86 - protein, 38 aa, Artificial Sequence
  variant of the indicator motif
DPEPGRCRRTDGKKWRCARDAHPDSKYCEKHMHRGKNR

SEQ ID NO: 87 - protein, 38 aa, Artificial Sequence
  variant of the indicator motif
DPEPGRCRRTDGKKWRCSKDAHPDSKYCEKHMHRGKNR

SEQ ID NO: 88 - protein, 38 aa, Artificial Sequence
  variant of the indicator motif
DPEPGRCRRTDGKKWRCAKDAHPDSKYCEKHMHRGKNR

SEQ ID NO: 89 - protein, 38 aa, Artificial Sequence
  variant of the indicator motif
DPEPGRCRRTDGKKWRCSREAYPDSKYCERHMHRGKNR

SEQ ID NO: 90 - protein, 38 aa, Artificial Sequence
  variant of the indicator motif
DPEPGRCRRTDGKKWRCAREAYPDSKYCERHMHRGKNR

SEQ ID NO: 91 - protein, 38 aa, Artificial Sequence
  variant of the indicator motif
DPEPGRCRRTDGKKWRCSKEAYPDSKYCERHMHRGKNR

SEQ ID NO: 92 - protein, 38 aa, Artificial Sequence
  variant of the indicator motif
DPEPGRCRRTDGKKWRCAKEAYPDSKYCERHMHRGKNR

SEQ ID NO: 93 - protein, 38 aa, Artificial Sequence
  variant of the indicator motif
DPEPGRCRRTDGKKWRCSRDAYPDSKYCERHMHRGKNR

SEQ ID NO: 94 - protein, 38 aa, Artificial Sequence
  variant of the indicator motif
DPEPGRCRRTDGKKWRCARDAYPDSKYCERHMHRGKNR

SEQ ID NO: 95 - protein, 38 aa, Artificial Sequence
  variant of the indicator motif
DPEPGRCRRTDGKKWRCSKDAYPDSKYCERHMHRGKNR

SEQ ID NO: 96 - protein, 38 aa, Artificial Sequence
  variant of the indicator motif
DPEPGRCRRTDGKKWRCAKDAYPDSKYCERHMHRGKNR

SEQ ID NO: 97 - protein, 38 aa, Artificial Sequence
  variant of the indicator motif
DPEPGRCRRTDGKKWRCSREAHPDSKYCERHMHRGKNR

SEQ ID NO: 98 - protein, 38 aa, Artificial Sequence
  variant of the indicator motif
DPEPGRCRRTDGKKWRCAREAHPDSKYCERHMHRGKNR

SEQ ID NO: 99 - protein, 38 aa, Artificial Sequence
  variant of the indicator motif
DPEPGRCRRTDGKKWRCSKEAHPDSKYCERHMHRGKNR

SEQ ID NO: 100 - protein, 38 aa, Artificial Sequence
  variant of the indicator motif
DPEPGRCRRTDGKKWRCAKEAHPDSKYCERHMHRGKNR

SEQ ID NO: 101 - protein, 38 aa, Artificial Sequence
  variant of the indicator motif
DPEPGRCRRTDGKKWRCSRDAHPDSKYCERHMHRGKNR

SEQ ID NO: 102 - protein, 38 aa, Artificial Sequence
  variant of the indicator motif
DPEPGRCRRTDGKKWRCARDAHPDSKYCERHMHRGKNR

SEQ ID NO: 103 - protein, 38 aa, Artificial Sequence
  variant of the indicator motif
DPEPGRCRRTDGKKWRCSKDAHPDSKYCERHMHRGKNR

SEQ ID NO: 104 - protein, 38 aa, Artificial Sequence
  variant of the indicator motif
DPEPGRCRRTDGKKWRCAKDAHPDSKYCERHMHRGKNR

SEQ ID NO: 105 - DNA, 1080 bp, Artificial Sequence
  cDNA of GmGRF5
atgatgagtgcaagtgcaggtgcaagaaataggtctccgttcacacaaattcagtggcaagagcttgagcaacaagctcttgtttttaagtacatggttacaggaacacctatcccaccagatctcatctactctattaaaagaagtctagacacttcaatttcttcaaggctcttcccacatcatccaattgggtggggatgttttgaaatgggatttggcagaaaagtagacccagagccagggaggtgcagaagaacagatggcaagaaatggagatgttcaaaggaggcatatccagactcaaagtactgtgaaagacacatgcacagaggcagaaaccgttcaagaaagcctgtggaagtttcttcagcaacaagcaccgccacaaacacctcccaaacaatcccatcatcttataccagaaacctttccttgaccaataacagtaaccccaacataacaccaccaccaccaccctcttctttccctttctctcatttgccctcttctatgcctattgatcagtcccaacccttttcccaatcctaccaaaactcttctctcaatcccttcttctactcccaatcaacctcctctagacccccagatgctgattttccaccccaagatgccaccacccaccacctattcatggactctgctggctcttattctcatgatgaaaagaattataggcatgttcatggaataagggaagatgtggatgagagagctttcttcccagaagcatcaggatcagctaggagctatacagactcgtaccaacaactatcaatgagctcctacaagtcctattcaaactccaactttcagaacattaataatgatgccaccaccaacccaagacagcaagagcagcaactacaacaacaacaacactgttttgttttagggacagacttcaaatcaacaaggccaagcaaagagaaagaagctgagacaacaacaggtcagagaccccttcaccgtttctttggggagtggccaccaaagaacacaacaacagattcctggctagatcttgcttccaactccagaatccaaaccgatgaatga

SEQ ID NO: 106 - protein, 359 aa, Glycine max
MMSASAGARNRSPFTQIQWQELEQQALVFKYMVTGTPIPPDLIYSIKRSLDTSISSRLFPHHPIGWGCFEMGFGRKVDPEPGRCRRTDGKKWRCSKEAYPDSKYCERHMHRGRNRSRKPVEVSSATSTATNTSQTIPSSYTRNLSLTNNSNPNITPPPPPSSFPFSHLPSSMPIDQSQPFSQSYQNSSLNPFFYSQSTSSRPPDADFPPQDATTHHLFMDSAGSYSHDEKNYRHVHGIREDVDERAFFPEASGSARSYTDSYQQLSMSSYKSYSNSNFQNINNDATTNPRQQEQQLQQQQHCFVLGTDFKSTRPSKEKEAETTTGQRPLHRFFGEWPPKNTTTDSWLDLASNSRIQTDE

SEQ ID NO: 107 - DNA, 1173 bp, Artificial Sequence
  cDNA of BnGRF5
atgatgagtctaagtggaaatggtgggagaacaatagagaggcctccatttacaccaacacaatggcaagaactggagaatcaagccctaatttacaagtacatggtctcaggagttcctgtcccacctgagctcatcttctccattagaagaagcttggactcttccttggtctctagactcctccctcaccaatccattgggtggggatgctatcagatggggtttggtagaaaaccagatccagaaccaggaaggtgcagaagaacagatggtaagaaatggagatgctcaagagaagcatacccagattcaaagtactgtgaaaaacacatgcacagaggaaggaaccgtgccagaaaatctattgatcagaatcagacaactgctcctttaacatcaccatctctctctttccccaacaacaacaacccaagccctaccttgtcttcttcctcctctacttattcagcttcttcttcatctccttccattgatgcttacagtaatatcaataggcttggtgttggtaatagtaacagtagaggttacttcaacaaccattcccttgactatccttatcctttgtcctcacctaaacagcaacaacaacaacagactcttcatcatgcttctgctttgtctcttcaccaaaacgcatctactgcttctcagttcaatgccttagcttctgcaactgaccataaagacttcagatactttcaagggattggggagagagttggagttggagctggggagaggactttttttccagaagcttctagaagctttcaagattctccataccatcaccaacaaccgttagctacagtaatgaatgacccgttccactctggtactgatcataaggttgatcatcagcatcacacatactcatccgtatcatcatcatctcagcatgatcaagatcatcatcgacaacaacagcagcaatgttttgttatgggcgctgacatgttcaacaaacccacaagaactgtcttcgcaaactcatctagacaagatcatcaagaagaggaggagaaagattcatcagaaacaaagaagtctctacatcatttctttggtgaggactgggcacagaacaaaaacagttcagattcttggcttgacctttcttcccattcaagactggacactggtagttga

SEQ ID NO: 108 - protein, 390 aa, Brassica napus
MMSLSGNGGRTIERPPFTPTQWQELENQALIYKYMVSGVPVPPELIFSIRRSLDSSLVSRLLPHQSIGWGCYQMGFGRKPDPEPGRCRRTDGKKWRCSREAYPDSKYCEKHMHRGRNRARKSIDQNQTTAPLTSPSLSFPNNNNPSPTLSSSSSTYSASSSSPSIDAYSNINRLGVGNSNSRGYFNNHSLDYPYPLSSPKQQQQQQTLHHASALSLHQNASTASQFNALASATDHKDFRYFQGIGERVGVGAGERTFFPEASRSFQDSPYHHQQPLATVMNDPFHSGTDHKVDHQHHTYSSVSSSSQHDQDHHRQQQQQCFVMGADMFNKPTRTVFANSSRQDHQEEEEKDSSETKKSLHHFFGEDWAQNKNSSDSWLDLSSHSRLDTGS

SEQ ID NO: 109 - DNA, 981 bp, Artificial Sequence
  cDNA of HaGRF5
atgatgatgatgagtactacaagcagtaaccaaaatccaaatgtgttcacagcatcacaatgggaagaactggaacagcaagctttaatctacaagtatatggtttcaggtgttccagttccaactgatctcatcttgtctgtcagaagaagtttgtataacacctcagcttcatcactatctaaccaacacacctcctccttaggaatatgggaagctggatcaagctttccatacaatcagttgtatcagattggtgggtatggtggcagaaagatagatttagaaccaggaagatgcagaagaacagatggaaaaaaatggaggtgctctaaagaagcttaccccgattcaaaatactgcgagagacacatgcacagaggtagaaaccgttcaagaaagcctgtggaattctcttcttcttcttcttcatcttcatctgctgccacaagtgttaataatgtttcttcttcatcagcaatctccaaatcaatcgatgcttaccctcctcctttctcaacttttatggattcttcatcttattctcaccaaacccttaaagattacaggcagatgcaaggaatgaaggatttaggagaggatgagagatcatcagcagcagcagcagcttactttcaactaaatgatccttacaccgccactacacaatctggtcaacaaaactactctcatttcagttttcaaaacctgaaagatgagcagaagaaggagcaagggcagcactgttttgtgatgggtactgatttcataaagccatcagaagaacatgaacccaccaaatccactaccacaaaagttaatgaaaccaccagtaaacaaccattccaccacttcttttcaccaccaaaagccacactgcttaaccctaaccatgacccaaactggggtgaagttgaccacccaaaggcccctttgtccacccaagaccttttccaatccaaaccaagaccttactggtag

SEQ ID NO: 110 - protein, 326 aa, Helianthus annuus
MMMMSTTSSNQNPNVFTASQWEELEQQALIYKYMVSGVPVPTDLILSVRRSLYNTSASSLSNQHTSSLGIWEAGSSFPYNQLYQIGGYGGRKIDLEPGRCRRTDGKKWRCSKEAYPDSKYCERHMHRGRNRSRKPVEFSSSSSSSSSAATSVNNVSSSSAISKSIDAYPPPFSTFMDSSSYSHQTLKDYRQMQGMKDLGEDERSSAAAAAYFQLNDPYTATTQSGQQNYSHFSFQNLKDEQKKEQGQHCFVMGTDFIKPSEEHEPTKSTTTKVNETTSKQPFHHFFSPPKATLLNPNHDPNWGEVDHPKAPLSTQDLFQSKPRPYW

SEQ ID NO: 111 - DNA, 1131 bp, Artificial Sequence
  cDNA of ZmGRF5
atgatgatgatgagcggtcgagcggccaccgcggggcggtacccgttcacggcgtcgcagtggcaggagctggagcaccaggcgctcatctacaagtgcctggcgtccggcaagcccatcccgtcctacctcatgccaccgctccgccgcatcctcgactccgccctcgccacgtcgccgtcgctcgccgccttcccgccgcaaccctcgctggggtgggggggctgcttcgggatgggcttcagcaggaagcccgccgacgaggacccggagcccgggcggtgccggcgcacggacggcaagaagtggcgctgctccaaggaggcgtacccggactccaagtactgcgagaagcacatgcaccggggcaagaaccgttcaagaaagcctgtggaaatgtccttggccacgccggcgccggcctcctccgccacaagcgccgccgccgccgccacctcctcgtcccaggcgccgtcctaccacagcccggcccccgccgtgccgtaccacgcgccctacggcgccgcgtaccatcacacgcagacgcaggtgacgatgagccccttccacctcctccacctcgagaccacccacccgcacccgccgccgccgccgccgccgccctactactacgcggaccagagggactacgcctacggcaaggaggtcggcgagcgcgccttcttctccgacggcgcgggcgagagggaccggcagcagcaggccgcggggcagtggcagttcaagcagctcgggacgatggaggcgacgaagcagccgtgcaccacgccgctgctcgtccccgccgccgggtacggccacggcgcggcgtcgccgtacggcgtcggtcaggccaaggaagacgaggaggaggaggaaacgcggcggcagcagcagcactgcttcgttcttggcgccgacctgcggctggcggagcggccgtcgggggcacatgacgccgccgcgcagaagccgctccggcatttcatcgacgagtggccgcacgagaaggggagcaataaggcggggtcgtggatgggggggctcgacggcgagacgacgcagctctccatgtctatcccgatggcggccgctgccgacctccccgtcacctcccgctaccgtacgtga

SEQ ID NO: 112 - protein, 376 aa, Zea mays
MMMMSGRAATAGRYPFTASQWQELEHQALIYKCLASGKPIPSYLMPPLRRILDSALATSPSLAAFPPQPSLGWGGCFGMGFSRKPADEDPEPGRCRRTDGKKWRCSKEAYPDSKYCEKHMHRGKNRSRKPVEMSLATPAPASSATSAAAAATSSSQAPSYHSPAPAVPYHAPYGAAYHHTQTQVTMSPFHLLHLETTHPHPPPPPPPPYYYADQRDYAYGKEVGERAFFSDGAGERDRQQQAAGQWQFKQLGTMEATKQPCTTPLLVPAAGYGHGAASPYGVGQAKEDEEEEETRRQQQHCFVLGADLRLAERPSGAHDAAAQKPLRHFIDEWPHEKGSNKAGSWMGGLDGETTQLSMSIPMAAAADLPVTSRYRT

SEQ ID NO: 113 - protein, 38 aa, Artificial Sequence
  variant of the indicator motif
DLEPGRCRRTDGKKWRCSREAYPDSKYCEKHMHRGRNR

SEQ ID NO: 114 - protein, 38 aa, Artificial Sequence
  variant of the indicator motif
DLEPGRCRRTDGKKWRCAREAYPDSKYCEKHMHRGRNR

SEQ ID NO: 115 - protein, 38 aa, Artificial Sequence
  variant of the indicator motif
DLEPGRCRRTDGKKWRCSKEAYPDSKYCEKHMHRGRNR

SEQ ID NO: 116 - protein, 38 aa, Artificial Sequence
  variant of the indicator motif
DLEPGRCRRTDGKKWRCAKEAYPDSKYCEKHMHRGRNR

SEQ ID NO: 117 - protein, 38 aa, Artificial Sequence
  variant of the indicator motif
DLEPGRCRRTDGKKWRCSRDAYPDSKYCEKHMHRGRNR

SEQ ID NO: 118 - protein, 38 aa, Artificial Sequence
  variant of the indicator motif
DLEPGRCRRTDGKKWRCARDAYPDSKYCEKHMHRGRNR

SEQ ID NO: 119 - protein, 38 aa, Artificial Sequence
  variant of the indicator motif
DLEPGRCRRTDGKKWRCSKDAYPDSKYCEKHMHRGRNR

SEQ ID NO: 120 - protein, 38 aa, Artificial Sequence
  variant of the indicator motif
DLEPGRCRRTDGKKWRCAKDAYPDSKYCEKHMHRGRNR

SEQ ID NO: 121 - protein, 38 aa, Artificial Sequence
  variant of the indicator motif
DLEPGRCRRTDGKKWRCSREAHPDSKYCEKHMHRGRNR

SEQ ID NO: 122 - protein, 38 aa, Artificial Sequence
  variant of the indicator motif
DLEPGRCRRTDGKKWRCAREAHPDSKYCEKHMHRGRNR

SEQ ID NO: 123 - protein, 38 aa, Artificial Sequence
  variant of the indicator motif
DLEPGRCRRTDGKKWRCSKEAHPDSKYCEKHMHRGRNR

SEQ ID NO: 124 - protein, 38 aa, Artificial Sequence
  variant of the indicator motif
DLEPGRCRRTDGKKWRCAKEAHPDSKYCEKHMHRGRNR

SEQ ID NO: 125 - protein, 38 aa, Artificial Sequence
  variant of the indicator motif
DLEPGRCRRTDGKKWRCSRDAHPDSKYCEKHMHRGRNR

SEQ ID NO: 126 - protein, 38 aa, Artificial Sequence
  variant of the indicator motif
DLEPGRCRRTDGKKWRCARDAHPDSKYCEKHMHRGRNR

SEQ ID NO: 127 - protein, 38 aa, Artificial Sequence
  variant of the indicator motif
DLEPGRCRRTDGKKWRCSKDAHPDSKYCEKHMHRGRNR

SEQ ID NO: 128 - protein, 38 aa, Artificial Sequence
  variant of the indicator motif
DLEPGRCRRTDGKKWRCAKDAHPDSKYCEKHMHRGRNR

SEQ ID NO: 129 - protein, 38 aa, Artificial Sequence
  variant of the indicator motif
DLEPGRCRRTDGKKWRCSREAYPDSKYCERHMHRGRNR

SEQ ID NO: 130 - protein, 38 aa, Artificial Sequence
  variant of the indicator motif
DLEPGRCRRTDGKKWRCAREAYPDSKYCERHMHRGRNR

SEQ ID NO: 131 - protein, 38 aa, Artificial Sequence
  variant of the indicator motif
DLEPGRCRRTDGKKWRCSKEAYPDSKYCERHMHRGRNR

SEQ ID NO: 132 - protein, 38 aa, Artificial Sequence
  variant of the indicator motif
DLEPGRCRRTDGKKWRCAKEAYPDSKYCERHMHRGRNR

SEQ ID NO: 133 - protein, 38 aa, Artificial Sequence
  variant of the indicator motif
DLEPGRCRRTDGKKWRCSRDAYPDSKYCERHMHRGRNR

SEQ ID NO: 134 - protein, 38 aa, Artificial Sequence
  variant of the indicator motif
DLEPGRCRRTDGKKWRCARDAYPDSKYCERHMHRGRNR

SEQ ID NO: 135 - protein, 38 aa, Artificial Sequence
  variant of the indicator motif
DLEPGRCRRTDGKKWRCSKDAYPDSKYCERHMHRGRNR

SEQ ID NO: 136 - protein, 38 aa, Artificial Sequence
  variant of the indicator motif
DLEPGRCRRTDGKKWRCAKDAYPDSKYCERHMHRGRNR

SEQ ID NO: 137 - protein, 38 aa, Artificial Sequence
  variant of the indicator motif
DLEPGRCRRTDGKKWRCSREAHPDSKYCERHMHRGRNR

SEQ ID NO: 138 - protein, 38 aa, Artificial Sequence
  variant of the indicator motif
DLEPGRCRRTDGKKWRCAREAHPDSKYCERHMHRGRNR

SEQ ID NO: 139 - protein, 38 aa, Artificial Sequence
  variant of the indicator motif
DLEPGRCRRTDGKKWRCSKEAHPDSKYCERHMHRGRNR

SEQ ID NO: 140 - protein, 38 aa, Artificial Sequence
  variant of the indicator motif
DLEPGRCRRTDGKKWRCAKEAHPDSKYCERHMHRGRNR

SEQ ID NO: 141 - protein, 38 aa, Artificial Sequence
  variant of the indicator motif
DLEPGRCRRTDGKKWRCSRDAHPDSKYCERHMHRGRNR

SEQ ID NO: 142 - protein, 38 aa, Artificial Sequence
  variant of the indicator motif
DLEPGRCRRTDGKKWRCARDAHPDSKYCERHMHRGRNR

SEQ ID NO: 143 - protein, 38 aa, Artificial Sequence
  variant of the indicator motif
DLEPGRCRRTDGKKWRCSKDAHPDSKYCERHMHRGRNR

SEQ ID NO: 144 - protein, 38 aa, Artificial Sequence
  variant of the indicator motif
DLEPGRCRRTDGKKWRCAKDAHPDSKYCERHMHRGRNR

SEQ ID NO: 145 - protein, 38 aa, Artificial Sequence
  variant of the indicator motif
DLEPGRCRRTDGKKWRCSREAYPDSKYCEKHMHRGKNR

SEQ ID NO: 146 - protein, 38 aa, Artificial Sequence
  variant of the indicator motif
DLEPGRCRRTDGKKWRCAREAYPDSKYCEKHMHRGKNR

SEQ ID NO: 147 - protein, 38 aa, Artificial Sequence
  variant of the indicator motif
DLEPGRCRRTDGKKWRCSKEAYPDSKYCEKHMHRGKNR

SEQ ID NO: 148 - protein, 38 aa, Artificial Sequence
  variant of the indicator motif
DLEPGRCRRTDGKKWRCAKEAYPDSKYCEKHMHRGKNR

SEQ ID NO: 149 - protein, 38 aa, Artificial Sequence
  variant of the indicator motif
DLEPGRCRRTDGKKWRCSRDAYPDSKYCEKHMHRGKNR

SEQ ID NO: 150 - protein, 38 aa, Artificial Sequence
  variant of the indicator motif
DLEPGRCRRTDGKKWRCARDAYPDSKYCEKHMHRGKNR

SEQ ID NO: 151 - protein, 38 aa, Artificial Sequence
  variant of the indicator motif
DLEPGRCRRTDGKKWRCSKDAYPDSKYCEKHMHRGKNR

SEQ ID NO: 152 - protein, 38 aa, Artificial Sequence
  variant of the indicator motif
DLEPGRCRRTDGKKWRCAKDAYPDSKYCEKHMHRGKNR

SEQ ID NO: 153 - protein, 38 aa, Artificial Sequence
  variant of the indicator motif
DLEPGRCRRTDGKKWRCSREAHPDSKYCEKHMHRGKNR

SEQ ID NO: 154 - protein, 38 aa, Artificial Sequence
  variant of the indicator motif
DLEPGRCRRTDGKKWRCAREAHPDSKYCEKHMHRGKNR

SEQ ID NO: 155 - protein, 38 aa, Artificial Sequence
  variant of the indicator motif
DLEPGRCRRTDGKKWRCSKEAHPDSKYCEKHMHRGKNR

SEQ ID NO: 156 - protein, 38 aa, Artificial Sequence
  variant of the indicator motif
DLEPGRCRRTDGKKWRCAKEAHPDSKYCEKHMHRGKNR

SEQ ID NO: 157 - protein, 38 aa, Artificial Sequence
  variant of the indicator motif
DLEPGRCRRTDGKKWRCSRDAHPDSKYCEKHMHRGKNR

SEQ ID NO: 158 - protein, 38 aa, Artificial Sequence
  variant of the indicator motif
DLEPGRCRRTDGKKWRCARDAHPDSKYCEKHMHRGKNR

SEQ ID NO: 159 - protein, 38 aa, Artificial Sequence
  variant of the indicator motif
DLEPGRCRRTDGKKWRCSKDAHPDSKYCEKHMHRGKNR

SEQ ID NO: 160 - protein, 38 aa, Artificial Sequence
  variant of the indicator motif
DLEPGRCRRTDGKKWRCAKDAHPDSKYCEKHMHRGKNR

SEQ ID NO: 161 - protein, 38 aa, Artificial Sequence
  variant of the indicator motif
DLEPGRCRRTDGKKWRCSREAYPDSKYCERHMHRGKNR

SEQ ID NO: 162 - protein, 38 aa, Artificial Sequence
  variant of the indicator motif
DLEPGRCRRTDGKKWRCAREAYPDSKYCERHMHRGKNR

SEQ ID NO: 163 - protein, 38 aa, Artificial Sequence
  variant of the indicator motif
DLEPGRCRRTDGKKWRCSKEAYPDSKYCERHMHRGKNR

SEQ ID NO: 164 - protein, 38 aa, Artificial Sequence
  variant of the indicator motif
DLEPGRCRRTDGKKWRCAKEAYPDSKYCERHMHRGKNR

SEQ ID NO: 165 - protein, 38 aa, Artificial Sequence
  variant of the indicator motif
DLEPGRCRRTDGKKWRCSRDAYPDSKYCERHMHRGKNR

SEQ ID NO: 166 - protein, 38 aa, Artificial Sequence
  variant of the indicator motif
DLEPGRCRRTDGKKWRCARDAYPDSKYCERHMHRGKNR

SEQ ID NO: 167 - protein, 38 aa, Artificial Sequence
  variant of the indicator motif
DLEPGRCRRTDGKKWRCSKDAYPDSKYCERHMHRGKNR

SEQ ID NO: 168 - protein, 38 aa, Artificial Sequence
  variant of the indicator motif
DLEPGRCRRTDGKKWRCAKDAYPDSKYCERHMHRGKNR

SEQ ID NO: 169 - protein, 38 aa, Artificial Sequence
  variant of the indicator motif
DLEPGRCRRTDGKKWRCSREAHPDSKYCERHMHRGKNR

SEQ ID NO: 170 - protein, 38 aa, Artificial Sequence
  variant of the indicator motif
DLEPGRCRRTDGKKWRCAREAHPDSKYCERHMHRGKNR

SEQ ID NO: 171 - protein, 38 aa, Artificial Sequence
  variant of the indicator motif
DLEPGRCRRTDGKKWRCSKEAHPDSKYCERHMHRGKNR

SEQ ID NO: 172 - protein, 38 aa, Artificial Sequence
  variant of the indicator motif
DLEPGRCRRTDGKKWRCAKEAHPDSKYCERHMHRGKNR

SEQ ID NO: 173 - protein, 38 aa, Artificial Sequence
  variant of the indicator motif
DLEPGRCRRTDGKKWRCSRDAHPDSKYCERHMHRGKNR

SEQ ID NO: 174 - protein, 38 aa, Artificial Sequence
  variant of the indicator motif
DLEPGRCRRTDGKKWRCARDAHPDSKYCERHMHRGKNR

SEQ ID NO: 175 - protein, 38 aa, Artificial Sequence
  variant of the indicator motif
DLEPGRCRRTDGKKWRCSKDAHPDSKYCERHMHRGKNR

SEQ ID NO: 176 - protein, 38 aa, Artificial Sequence
  variant of the indicator motif
DLEPGRCRRTDGKKWRCAKDAHPDSKYCERHMHRGKNR

SEQ ID NO: 177 - protein, 38 aa, Artificial Sequence
  GRF5 specific indicator motif
  VARIANT (2)..(2): X is proline (P) or leucine (L)
  VARIANT (18)..(18): X is serine (S) or alanine (A)
  VARIANT (19)..(19): X is arginine (R) or lysine (K)
  VARIANT (20)..(20): X is glutamic acid (E) or aspartic acid (D)
  VARIANT (22)..(22): X is tyrosine (Y) or histidine (H)
  VARIANT (30)..(30): X is lysine (K) or arginine (R)
  VARIANT (36)..(36): X is arginine (R) or lysine (K)
DXEPGRCRRTDGKKWRCXXXAXPDSKYCEXHMHRGXNR

SEQ ID NO: 178 - protein, 38 aa, Arabidopsis thaliana
DPEPGRCRRTDGKKWRCSRDAVPDQKYCERHINRGRHR

SEQ ID NO: 179 - protein, 38 aa, Arabidopsis thaliana; identical to SEQ ID NO: 178

SEQ ID NO: 180 - protein, 38 aa, Arabidopsis thaliana
DPEPGRCRRTDGKKWRCSRDVFAGHKYCERHMHRGRNR

SEQ ID NO: 181 - protein, 38 aa, Arabidopsis thaliana
DPEPGRCKRTDGKKWRCSRDVVAGHKYCDRHIHRGRNR

SEQ ID NO: 182 - protein, 38 aa, Arabidopsis thaliana
DAEPGRCRRTDGKKWRCSKEAYPDSKYCERHMHRGKNR

SEQ ID NO: 183 - protein, 38 aa, Arabidopsis thaliana
DLEPGRCRRTDGKKWRCAKEVVSNHKYCEKHLHRGRPR

SEQ ID NO: 184 - protein, 38 aa, Arabidopsis thaliana
DLEPWRCKRTDGKKWRCSRNVIPDQKYCERHTHKSRPR

SEQ ID NO: 185 - protein, 38 aa, Arabidopsis thaliana
ETEPTRCRRTDGKKWRCSNTVLLFEKYCERHMHRGRKR

SEQ ID NO: 186 - protein, 38 aa, Arabidopsis thaliana; identical to SEQ ID NO: 41

SEQ ID NO: 187 - protein, 38 aa, Beta vulgaris; identical to SEQ ID NO: 91

SEQ ID NO: 188 - protein, 38 aa, Zea mays; identical to SEQ ID NO: 75

SEQ ID NO: 189 - protein, 38 aa, Triticum aestivum; identical to SEQ ID NO: 75

SEQ ID NO: 190 - protein, 38 aa, Brassica napus; identical to SEQ ID NO: 41

SEQ ID NO: 191 - protein, 38 aa, Brassica rapa; identical to SEQ ID NO: 49

SEQ ID NO: 192 - protein, 38 aa, Brassica oleracea; identical to SEQ ID NO: 41

SEQ ID NO: 193 - protein, 38 aa, Raphanus sativus; identical to SEQ ID NO: 41

SEQ ID NO: 194 - protein, 38 aa, Sorghum bicolor; identical to SEQ ID NO: 75

SEQ ID NO: 195 - protein, 38 aa, Helianthus annuus; identical to SEQ ID NO: 59

SEQ ID NO: 196 - protein, 38 aa, Solanum tuberosum; identical to SEQ ID NO: 64

SEQ ID NO: 197 - protein, 38 aa, Hordeum vulgare; identical to SEQ ID NO: 73

SEQ ID NO: 198 - protein, 38 aa, Secale cereale; identical to SEQ ID NO: 75

SEQ ID NO: 199 - protein, 38 aa, Glycine max; identical to SEQ ID NO: 59

SEQ ID NO: 200 - protein, 38 aa, Gossypium hirsutum; identical to SEQ ID NO: 59

SEQ ID NO: 201 - protein, 38 aa, Oryza sativa; identical to SEQ ID NO: 75

SEQ ID NO: 202 - protein, 38 aa, Glycine max; identical to SEQ ID NO: 59

SEQ ID NO: 203 - protein, 38 aa, Brassica napus; identical to SEQ ID NO: 41

SEQ ID NO: 204 - protein, 38 aa, Helianthus annuus; identical to SEQ ID NO: 131

SEQ ID NO: 205 - protein, 38 aa, Zea mays; identical to SEQ ID NO: 75

SEQ ID NO: 206 - protein, 38 aa, Zea mays; identical to SEQ ID NO: 75

SEQ ID NO: 207 - DNA, 1143 bp, Artificial Sequence
  synthetic DNA encoding BvGRF5 protein of SEQ ID NO: 4
atgtctactgctacagctactgttggaggcggaggtggtggtggaagatctaagtttcctttcacggcgacccaatggcaagagcttgaacatcaggctctcatctacaagtacatggctgctggtgtgcctattcctcctgatctcttgttcaccatcaagcgtagcctcgacagcagcctctcttctaaactcttcccataccagccttcaccgcttggatggaacccttaccaaatgggatacgggaagaagatcgatcctgagcctggaagatgtaggcgtaccgatggaaaaaagtggcgttgcagcaaagaggcttacccggattctaagtactgcgagagacacatgcaccgtgggaagaacagatctaggaagcctgttgagtctccgctcactactacttctaccaccgtgtcgaacaataacaacaacaacaacaataacaacaactccgccgccaactcctctctcactgttgctgctgctgcagctgccgcttctcttactaatcagtcactcctcaacaagaacccgtcctccgtgtctactagccttttcagccttccgtcctctgacagctcttgcaactctcatcttctctacccgcactccagctacaaccacaaggattacagagagaggtactaccaggggctcaaagaagaagttggagagcacgccttcttcaccgagtcatctggatcttctatgcgtgggttcagcgggtcatctatggatgagtcttggcaaatcggcggagggtctaacatcgatcatcatcaacagcaacagcagcagtccaagcagtctggtggataccctaactaccttcagcagctccagtctaacagcaccacctctaacaacggaaccagcgctaagcaagagaagcagtgttacatctggggccgtgatttcaactgcgacctctctatgaaggtcgaagaggaacgtgagaacttccacgaaaagacgacccaccacttcttcgatgagtggcctatcaaatctggtggacgtggtggtagggattcttcttggcacgatagcagctctactacccagctctctatcagcatcccgtcctctacttctcatcaccacgactttttcttgaccaactcgcgagacagctga

SEQ ID NO: 208 - DNA, 1206 bp, Artificial Sequence
  synthetic DNA encoding ZmGRF5 protein according to SEQ ID NO: 209
atgatgatgatgtcatctggtagagctggcggcggtgctaccgctggtagatacccattcaccgccagccagtggcaagagcttgagcaccaggcgctgatctacaagtgcctggctagcggcaagccgattccgagctacctgatgccaccactgaggcgcatcctggactctgctctggctacctctccaagcctggcttacccaccacagccatctcttggttggggctgcttcggcatgggcttcactagaaaggctgacgaggatccagagcctggtaggtgcagaaggaccgacggtaagaagtggcgctgcagcaaagaggcttacccggacagcaagtactgcgagaagcacatgcacaggggcaagaacaggtcccgcaagccagttgagatgagcctcgctactcctgctccggcaccagctccagctgctgctactaccgctactgctaccagctctccggctccatcttaccacaggccagctcacgatgctaccccatctccataccacgctctgtacggcggaggcggtggtggcggtggctctccttactctgcttctgctaggccaggcgctacaggtggtggtggggcttaccatcatgctcagcacgtgagcccattccacctccacctcgagactacccatccgcatcctccgccgccatacaactactctgctgaccagagggactacgcctacggccatgcagctgctaaagaggttggcgagcacgccttcttctctgatggtgctggtgagagggttgacaggcaggctgctgctggccaatggcagttcaggcaactgggcgtcgagactaagccgggtccaactccactgttcccagttgctggctacggtcacggtgctgcttctccatacggcgttgagatgggcaaagacgacgacgagcaagaggaaaggcgcaggcagcattgcttcgtgcttggcgctgacctgaggctcgagaggccatcttctggtcacggccacggccatgaccacgatgatgccgctgctgctcagaagccactcaggccattcttcgacgagtggccacaccagaagggcgacaaggctggttcttggatgggcctcgatggcgagactcagctgtccatgagcatcccaatggccgctaccgatctgccagtgacctctaggtttaggaacggcggccactacgagtga

SEQ ID NO: 209 - protein, 401 aa, Zea mays
MMMMSSGRAGGGATAGRYPFTASQWQELEHQALIYKCLASGKPIPSYLMPPLRRILDSALATSPSLAYPPQPSLGWGCFGMGFTRKADEDPEPGRCRRTDGKKWRCSKEAYPDSKYCEKHMHRGKNRSRKPVEMSLATPAPAPAPAAATTATATSSPAPSYHRPAHDATPSPYHALYGGGGGGGGSPYSASARPGATGGGGAYHHAQHVSPFHLHLETTHPHPPPPYNYSADQRDYAYGHAAAKEVGEHAFFSDGAGERVDRQAAAGQWQFRQLGVETKPGPTPLFPVAGYGHGAASPYGVEMGKDDDEQEERRRQHCFVLGADLRLERPSSGHGHGHDHDDAAAAQKPLRPFFDEWPHQKGDKAGSWMGLDGETQLSMSIPMAATDLPVTSRFRNGGHYE

SEQ ID NO: 210 - DNA, 1131 bp, Artificial Sequence
  synthetic DNA encoding ZmGRF5 protein of SEQ ID NO: 6
atgatgatgatgtctggcagggctgctaccgccggcagatacccattcactgctagccagtggcaagagcttgagcaccaggcgctgatctacaagtgcctggctagcggcaagccgattccgagctacctgatgccaccactgaggcgcatcctggactctgctctggctacctctccaagcctggctgcttttccaccacagccatctcttggttggggcggctgcttcggtatgggcttttctaggaagccagccgacgaggatccagagcctggtagatgtagaaggaccgacggcaagaagtggcgctgcagcaaagaggcttacccggacagcaagtactgcgagaagcacatgcacaggggcaagaacaggtcccgcaagccagttgagatgagcctggctactccagctccagctagcagcgctacatcagccgctgctgctgctacttctagctctcaggccccgtcctaccattcaccggctccagctgttccataccacgctccatacggcgctgcctaccaccatactcagacccaggtgaccatgtctccgttccatctgctgcacctcgagactacccatccgcatcctccgcctccgccacctccaccatattactacgctgaccagagggactacgcctacggcaaagaggttggcgagagggccttcttctctgatggtgctggtgagagggatcgccagcaacaagctgctggccaatggcagttcaagcagctgggcaccatggaagccaccaagcagccatgcactaccccactgcttgtgccagctgctggttacggtcatggcgccgcttcaccatacggtgttggccaggctaaagaggacgaggaagaagaggaaaccaggcgccagcagcaacactgcttcgtgctgggtgctgatctgaggcttgccgagaggccatctggcgctcatgatgccgctgctcagaagccactcaggcacttcattgacgagtggccgcacgagaagggctctaacaaggctggctcttggatgggcggcctggatggcgagactactcagctgtctatgagcatcccaatggccgctgccgctgatctgccagtgacttctaggtacaggacctga